European Patent Application EP 4 310 187 A1, published January 24, 2024. Title: Modified Human Serum Albumin-Thioredoxin Fusion Protein. Applicant: KM Biologics National University Corporation KUMAMOTO UNIVERSITY. The sequence listing filed with the application follows.

SEQUENCE LISTING (1 sequence)

SEQ ID NO: 1 - protein, 699 aa, Artificial sequence
  Human Serum Albumin-Thioredoxin Fusion Protein
DAHKSEVAHRFKDLGEENFKALVLIAFAQYLQQCPFEDHVKLVNEVTEFAKTCVADESAENCDKSLHTLFGDKLCTVATLRETYGEMADCCAKQEPERNECFLQHKDDNPNLPRLVRPEVDVMCTAFHDNEETFLKKYLYEIARRHPYFYAPELLFFAKRYKAAFTECCQAADKAACLLPKLDELRDEGKASSAKQRLKCASLQKFGERAFKAWAVARLSQRFPKAEFAEVSKLVTDLTKVHTECCHGDLLECADDRADLAKYICENQDSISSKLKECCEKPLLEKSHCIAEVENDEMPADLPSLAADFVESKDVCKNYAEAKDVFLGMFLYEYARRHPDYSVVLLLRLAKTYETTLEKCCAAADPHECYAKVFDEFKPLVEEPQNLIKQNCELFEQLGEYKFQNALLVRYTKKVPQVSTPTLVEVSRNLGKVGSKCCKHPEAKRMPCAEDYLSVVLNQLCVLHEKTPVSDRVTKCCTESLVNRRPCFSALEVDETYVPKEFNAETFTFHADICTLSEKERQIKKQTALVELVKHKPKATKEQLKAVMDDFAAFVEKCCKADDKETCFAEEGKKLVAASQAALGLGGGGSGGGGSVKQIESKTAFQEALDAAGDKLVVVDFSATWCGPCKMIKPFFHSLSEKYSNVIFLEVDVDDCQDVASECEVKCMPTFQFFKKGQKVGEFSGANKEKLEATINELV